European Patent Specification EP 3 455 375 B1, published March 13, 2024. Title: DETECTION OF MET EXON 14 DELETIONS AND ASSOCIATED THERAPIES. Applicant: Roche Diagnostics GmbH F. Hoffmann-La Roche AG Roche Molecular Systems, Inc. The sequence listing filed with the application follows.

SEQUENCE LISTING (55 sequences)

SEQ ID NO: 1 - DNA, 19 bp, Artificial Sequence
  source: /note="Description of Artificial Sequence: Synthetic primer"
ttgggtttttcctgtggct

SEQ ID NO: 2 - DNA, 19 bp, Artificial Sequence
  source: /note="Description of Artificial Sequence: Synthetic primer"
ttgggtttttcctgtggct

SEQ ID NO: 3 - DNA, 19 bp, Artificial Sequence
  source: /note="Description of Artificial Sequence: Synthetic primer"
  source: /note="Description of Combined DNA/RNA Molecule: Synthetic primer"
ttgggtttttcctgtggcu

SEQ ID NO: 4 - DNA, 19 bp, Artificial Sequence
  source: /note="Description of Artificial Sequence: Synthetic primer"
  source: /note="Description of Combined DNA/RNA Molecule: Synthetic primer"
ttgggtttttcctgtggcu

SEQ ID NO: 5 - DNA, 20 bp, Artificial Sequence
  source: /note="Description of Artificial Sequence: Synthetic primer"
cttgggtttttcctgtggct

SEQ ID NO: 6 - DNA, 21 bp, Artificial Sequence
  source: /note="Description of Artificial Sequence: Synthetic primer"
cttgggtttttcctgtggctg

SEQ ID NO: 7 - DNA, 18 bp, Artificial Sequence
  source: /note="Description of Artificial Sequence: Synthetic primer"
tgggtttttcctgtggct

SEQ ID NO: 8 - DNA, 20 bp, Artificial Sequence
  source: /note="Description of Artificial Sequence: Synthetic primer"
ttgggtttttcctgtggctg

SEQ ID NO: 9 - DNA, 23 bp, Artificial Sequence
  source: /note="Description of Artificial Sequence: Synthetic primer"
tcaaatgaatctgtagactaccg

SEQ ID NO: 10 - DNA, 23 bp, Artificial Sequence
  source: /note="Description of Artificial Sequence: Synthetic primer"
tcaaatgaatctgtagactaccg

SEQ ID NO: 11 - DNA, 23 bp, Artificial Sequence
  source: /note="Description of Artificial Sequence: Synthetic primer"
tcaaatgaatctgtagactaccg

SEQ ID NO: 12 - DNA, 23 bp, Artificial Sequence
  source: /note="Description of Artificial Sequence: Synthetic primer"
tcaaatgaatctgtagactaccg

SEQ ID NO: 13 - DNA, 26 bp, Artificial Sequence
  source: /note="Description of Artificial Sequence: Synthetic primer"
aatggtttcaaatgaatctgtagact

SEQ ID NO: 14 - DNA, 27 bp, Artificial Sequence
  source: /note="Description of Artificial Sequence: Synthetic primer"
aaatggtttcaaatgaatctgtagact

SEQ ID NO: 15 - DNA, 27 bp, Artificial Sequence
  source: /note="Description of Artificial Sequence: Synthetic primer"
agaaatggtttcaaatgaatctgtaga

SEQ ID NO: 16 - DNA, 27 bp, Artificial Sequence
  source: /note="Description of Artificial Sequence: Synthetic primer"
gaaatggtttcaaatgaatctgtagac

SEQ ID NO: 17 - DNA, 22 bp, Artificial Sequence
  source: /note="Description of Artificial Sequence: Synthetic primer"
gagtgtgtactcttgcatcgta

SEQ ID NO: 18 - DNA, 22 bp, Artificial Sequence
  source: /note="Description of Artificial Sequence: Synthetic primer"
  source: /note="Description of Combined DNA/RNA Molecule: Synthetic primer"
gagtgtgtactcttgcatcgua

SEQ ID NO: 19 - DNA, 22 bp, Artificial Sequence
  source: /note="Description of Artificial Sequence: Synthetic primer"
gagtgtgtactcttgcatcgta

SEQ ID NO: 20 - DNA, 22 bp, Artificial Sequence
  source: /note="Description of Artificial Sequence: Synthetic primer"
  source: /note="Description of Combined DNA/RNA Molecule: Synthetic primer"
gagtgtgtactcttgcatcgua

SEQ ID NO: 21 - DNA, 20 bp, Artificial Sequence
  source: /note="Description of Artificial Sequence: Synthetic primer"
agtgtgtactcttgcatcgt

SEQ ID NO: 22 - DNA, 22 bp, Artificial Sequence
  source: /note="Description of Artificial Sequence: Synthetic primer"
gagtgtgtactcttgcatcgta

SEQ ID NO: 23 - DNA, 21 bp, Artificial Sequence
  source: /note="Description of Artificial Sequence: Synthetic primer"
tgaggagtgtgtactcttgca

SEQ ID NO: 24 - DNA, 20 bp, Artificial Sequence
  source: /note="Description of Artificial Sequence: Synthetic primer"
gaggagtgtgtactcttgca

SEQ ID NO: 25 - DNA, 18 bp, Artificial Sequence
  source: /note="Description of Artificial Sequence: Synthetic primer"
tgcacttgtcggcatgaa

SEQ ID NO: 26 - DNA, 19 bp, Artificial Sequence
  source: /note="Description of Artificial Sequence: Synthetic primer"
ctgcacttgtcggcatgaa

SEQ ID NO: 27 - DNA, 19 bp, Artificial Sequence
  source: /note="Description of Artificial Sequence: Synthetic primer"
  source: /note="Description of Combined DNA/RNA Molecule: Synthetic primer"
ctgcacttgtcggcaugaa

SEQ ID NO: 28 - DNA, 19 bp, Artificial Sequence
  source: /note="Description of Artificial Sequence: Synthetic primer"
  source: /note="Description of Combined DNA/RNA Molecule: Synthetic primer"
ctgcacttgtcggcaugaa

SEQ ID NO: 29 - DNA, 19 bp, Artificial Sequence
  source: /note="Description of Artificial Sequence: Synthetic primer"
cttgtcggcatgaaccgtt

SEQ ID NO: 30 - DNA, 18 bp, Artificial Sequence
  source: /note="Description of Artificial Sequence: Synthetic primer"
ttgtcggcatgaaccgtt

SEQ ID NO: 31 - DNA, 18 bp, Artificial Sequence
  source: /note="Description of Artificial Sequence: Synthetic primer"
cttgtcggcatgaaccgt

SEQ ID NO: 32 - DNA, 19 bp, Artificial Sequence
  source: /note="Description of Artificial Sequence: Synthetic primer"
acttgtcggcatgaaccgt

SEQ ID NO: 33 - DNA, 19 bp, Artificial Sequence
  source: /note="Description of Artificial Sequence: Synthetic primer"
tgcacttgtcggcatgaac

SEQ ID NO: 34 - DNA, 19 bp, Artificial Sequence
  source: /note="Description of Artificial Sequence: Synthetic primer"
ctgcacttgtcggcatgaa

SEQ ID NO: 35 - DNA, 19 bp, Artificial Sequence
  source: /note="Description of Artificial Sequence: Synthetic primer"
gcacttgtcggcatgaacc

SEQ ID NO: 36 - DNA, 20 bp, Artificial Sequence
  source: /note="Description of Artificial Sequence: Synthetic primer"
ctgcacttgtcggcatgaac

SEQ ID NO: 37 - DNA, 20 bp, Artificial Sequence
  source: /note="Description of Artificial Sequence: Synthetic primer"
ttgtcggcatgaaccgttct

SEQ ID NO: 38 - DNA, 18 bp, Artificial Sequence
  source: /note="Description of Artificial Sequence: Synthetic primer"
gtcggcatgaaccgttct

SEQ ID NO: 39 - DNA, 34 bp, Artificial Sequence
  source: /note="Description of Artificial Sequence: Synthetic probe"
agaaagcaaattaaagatcagtttcctaattcat

SEQ ID NO: 40 - DNA, 34 bp, Artificial Sequence
  source: /note="Description of Artificial Sequence: Synthetic probe"
  source: /note="Description of Combined DNA/RNA Molecule: Synthetic probe"
agaaagcaaattaaagaucagtttcctaattcat

SEQ ID NO: 41 - DNA, 34 bp, Artificial Sequence; identical to SEQ ID NO: 40
  source: /note="Description of Artificial Sequence: Synthetic probe"
  source: /note="Description of Combined DNA/RNA Molecule: Synthetic probe"

SEQ ID NO: 42 - DNA, 34 bp, Artificial Sequence; identical to SEQ ID NO: 39
  source: /note="Description of Artificial Sequence: Synthetic probe"

SEQ ID NO: 43 - DNA, 34 bp, Artificial Sequence; identical to SEQ ID NO: 40
  source: /note="Description of Artificial Sequence: Synthetic probe"
  source: /note="Description of Combined DNA/RNA Molecule: Synthetic probe"

SEQ ID NO: 44 - DNA, 34 bp, Artificial Sequence
  source: /note="Description of Artificial Sequence: Synthetic probe"
agaaagcaaattaaagatctgggcagtgaattag

SEQ ID NO: 45 - DNA, 34 bp, Artificial Sequence
  source: /note="Description of Artificial Sequence: Synthetic probe"
  source: /note="Description of Combined DNA/RNA Molecule: Synthetic probe"
agaaagcaaattaaagauctgggcagtgaattag

SEQ ID NO: 46 - DNA, 34 bp, Artificial Sequence; identical to SEQ ID NO: 44
  source: /note="Description of Artificial Sequence: Synthetic probe"

SEQ ID NO: 47 - DNA, 35 bp, Artificial Sequence
  source: /note="Description of Artificial Sequence: Synthetic probe"
agctacttttccagaagatcagtttcctaattcat

SEQ ID NO: 48 - DNA, 35 bp, Artificial Sequence; identical to SEQ ID NO: 47
  source: /note="Description of Artificial Sequence: Synthetic probe"

SEQ ID NO: 49 - DNA, 35 bp, Artificial Sequence; identical to SEQ ID NO: 47
  source: /note="Description of Artificial Sequence: Synthetic probe"

SEQ ID NO: 50 - DNA, 35 bp, Artificial Sequence
  source: /note="Description of Artificial Sequence: Synthetic probe"
  source: /note="Description of Combined DNA/RNA Molecule: Synthetic probe"
agctacttttccagaagaucagtttcctaattcat

SEQ ID NO: 51 - DNA, 34 bp, Artificial Sequence; identical to SEQ ID NO: 40
  source: /note="Description of Artificial Sequence: Synthetic probe"
  source: /note="Description of Combined DNA/RNA Molecule: Synthetic probe"

SEQ ID NO: 52 - DNA, 35 bp, Artificial Sequence
  source: /note="Description of Artificial Sequence: Synthetic probe"
agcaaattaaagatcagtttcctaattcatctcag

SEQ ID NO: 53 - DNA, 34 bp, Artificial Sequence
  source: /note="Description of Artificial Sequence: Synthetic probe"
ttaaagatcagtttcctaattcatctcagaacgg

SEQ ID NO: 54 - DNA, 34 bp, Artificial Sequence
  source: /note="Description of Artificial Sequence: Synthetic probe"
  source: /note="Description of Combined DNA/RNA Molecule: Synthetic probe"
tuaaagatcagtttcctaattcatctcagaacgg

SEQ ID NO: 55 - DNA, 34 bp, Artificial Sequence
  source: /note="Description of Artificial Sequence: Synthetic probe"
aatttctagtcaaaggattaagtagagtcttgcc